European Patent Application EP 4 205 769 A1, published July 5, 2023. Title: ANTIGEN-BINDING CONSTRUCTS AND METHODS OF USE THEREOF. Applicant: Imaginab, Inc. Wilson, Ian Andrew Behera, Deepak Le, William Huy. The sequence listing filed with the application follows.

SEQUENCE LISTING (147 sequences)

SEQ ID NO: 1 - protein, 118 aa, Murine
EVQLQQSGAELVKPGASVKLSCTASGFNIKDTYIHFVRQRPEQGLEWIGRIDPANDNTLYASKFQGKATITADTSSNTAYMHLCSLTSGDTAVYYCGRGYGYYVFDHWGQGTTLTVSS

SEQ ID NO: 2 - protein, 120 aa, Homo sapiens [sequence omitted]

SEQ ID NO: 3 - protein, 118 aa, Artificial Sequence
  Antigen binding construct or fragment thereof
EVQLVESGGGLVQPGGSLRLSCAASGFNIKDTYIHWVRQAPGKGLEWVARIDPANDNTLYASKFQGRATISADTSKNTAYLQMNSLRAEDTAVYYCGRGYGYYVFDHWGQGTLVTVSS

SEQ ID NO: 4 - protein, 118 aa, Murine
QVQLQQSGAELVKPGASVKLSCTASGFNIKDTYIHFVRQRPEQGLEWIGRIDPANDNTLYASKFQGKATITADTSSNTAYMHLCSLTSGDTAVYYCGRGYGYYVFDHWGQGTTLTVSS

SEQ ID NO: 5 - protein, 115 aa, Homo sapiens
EVQLVQSGAEVKKPGATVKISCKVSGYTFTDYYMHWVQQAPGKGLEWMGLVDPEDGETIYAEKFQGRVTITADTSTDTAYMELSSLRSEDTAVYYCATAEYFQHWGQGTLVTVSS

SEQ ID NO: 6 - protein, 118 aa, Artificial Sequence
  Antigen binding construct or fragment thereof
QVQLVQSGAEVKKPGATVKISCKVSGFNIKDTYIHWVQQAPGKGLEWMGRIDPANDNTLYASKFQGRVTITADTSTDTAYMELSSLRSEDTAVYYCARGYGYYVFDHWGQGTLVTVSS

SEQ ID NO: 7 - protein, 107 aa, Murine
DVQINQSPSFLAASPGETITINCRTSRSISQYLAWYQEKPGKTNKLLIYSGSTLQSGIPSRFSGSGSGTDFTLTISGLEPEDFAMYYCQQHNENPLTFGAGTKLELK

SEQ ID NO: 8 - protein, 107 aa, Homo sapiens
DIQMTQSPSSLSASVGDRVTITCRASQGISNYLAWYQQKPGKVPKLLIYAASTLQSGVPSRFSGSGSGTDFTLTISSLQPEDVATYYCQKYNSAPLTFGGGTKVEIK

SEQ ID NO: 9 - protein, 107 aa, Artificial Sequence
  Antigen binding construct or fragment thereof
DVQITQSPSSLSASVGDRVTITCRTSRSISQYLAWYQQKPGKVPKLLIYSGSTLQSGVPSRFSGSGSGTDFTLTISSLQPEDVATYYCQQHNENPLTFGGGTKVEIK

SEQ ID NO: 10 - DNA, 768 bp, Artificial Sequence
  Antigen binding construct or fragment thereof
atggagaccgatacactgctgctgtgggtgctgctgctctgggtccctggcagcacaggagacatccagatgacacagagccctagctccctgagcgcttccgtgggagatagggtgaccatcacatgccggacctccaggtccatctcccagtacctggcctggtaccagcagaagcccggcaaggtgcccaagctgctcatctatagcggcagcaccctgcagagcggagtgccttcccggttttccggatccggctccggcacagactttaccctgaccatctccagcctgcagcctgaggatgtcgccacctactactgccaacagcacaacgagaaccccctgaccttcggcggcggaaccaaggtcgagatcaagggaggaggctccggaggaggaggccaagtgcagctggtccaatccggcgccgaagtgaaaaagcccggcgccaccgtgaagatcagctgcaaggtgtccggcttcaacatcaaggacacctatatccactgggtccagcaagcccccggaaaaggcctggagtggatgggacggattgaccccgccaacgacaacacactctatgcctccaagttccagggcagggtgacaatcaccgccgacaccagcaccgacacagcttatatggagctgtcctccctccggtccgaggataccgccgtctactactgcgccaggggctacggctactacgtgtttgaccactggggccagggcaccctggtgacagtgtccagcggaggctgc

SEQ ID NO: 11 - DNA, 768 bp, Artificial Sequence
  Antigen binding construct or fragment thereof
atggagaccgacaccctgctgctctgggtcctcctgctgtgggtgcctggcagcacaggacaggtgcaactggtgcagagcggcgccgaggtcaagaaacctggcgccaccgtgaagatcagctgcaaggtgtccggcttcaacatcaaggacacctacatccactgggtccaacaagcccccggaaagggcctggaatggatgggccggattgaccccgccaacgacaacaccctctatgccagcaagttccagggcagggtcaccatcaccgccgacaccagcaccgacaccgcctacatggagctgagcagcctgcggagcgaagacaccgccgtgtactactgcgccaggggctacggctactacgtcttcgaccattggggacagggcaccctcgtgacagtgtccagcggaggaggatccggcggaggaggagatatccagatgacccagagcccttccagcctgtccgcttccgtgggagatcgggtgaccatcacatgcaggacctccaggtccatctcccagtacctggcctggtaccaacagaagcccggcaaggtgcccaagctgctgatctacagcggcagcacactgcaatccggcgtcccttcccggttttccggatccggatccggcaccgacttcaccctgaccatcagctccctgcaacccgaggacgtggccacctactactgtcagcagcacaacgagaaccccctcacctttggcggcggaaccaaggtcgagatcaagggcggctgc

SEQ ID NO: 12 - protein, 253 aa, Artificial Sequence
  Antigen binding construct or fragment thereof
METDTLLLWVLLLWVPGSTGDIQMTQSPSSLSASVGDRVTITCRTSRSISQYLAWYQQKPGKVPKLLIYSGSTLQSGVPSRFSGSGSGTDFTLTISSLQPEDVATYYCQQHNENPLTFGGGTKVEIKSGGGGQVQLVQSGAEVKKPGATVKISCKVSGFNIKDTYIHWVQQAPGKGLEWMGRIDPANDNTLYASKFQGRVTITADTSTDTAYMELSSLRSEDTAVYYCARGYGYYVFDHWGQGTLVTVSSGGC

SEQ ID NO: 13 - protein, 253 aa, Artificial Sequence
  Antigen binding construct or fragment thereof
METDTLLLWVLLLWVPGSTGQVQLVQSGAEVKKPGATVKISCKVSGFNIKDTYIHWVQQAPGKGLEWMGRIDPANDNTLYASKFQGRVTITADTSTDTAYMELSSLRSEDTAVYYCARGYGYYVFDHWGQGTLVTVSSSGGGGDIQMTQSPSSLSASVGDRVTITCRTSRSISQYLAWYQQKPGKVPKLLIYSGSTLQSGVPSRFSGSGSGTDFTLTISSLQPEDVATYYCQQHNENPLTFGGGTKVEIKGGC

SEQ ID NO: 14 - protein, 256 aa, Artificial Sequence
  Antigen binding construct or fragment thereof
METDTLLLWVLLLWVPGSTGDIQMTQSPSSLSASVGDRVTITCRTSRSISQYLAWYQQKPGKVPKLLIYSGSTLQSGVPSRFSGSGSGTDFTLTISSLQPEDVATYYCQQHNENPLTFGGGTKVEIKGGGSGGGGQVQLVQSGAEVKKPGATVKISCKVSGFNIKDTYIHWVQQAPGKGLEWMGRIDPANDNTLYASKFQGRVTITADTSTDTAYMELSSLRSEDTAVYYCARGYGYYVFDHWGQGTLVTVSSGGC

SEQ ID NO: 15 - protein, 256 aa, Artificial Sequence
  Antigen binding construct or fragment thereof
METDTLLLWVLLLWVPGSTGQVQLVQSGAEVKKPGATVKISCKVSGFNIKDTYIHWVQQAPGKGLEWMGRIDPANDNTLYASKFQGRVTITADTSTDTAYMELSSLRSEDTAVYYCARGYGYYVFDHWGQGTLVTVSSGGGSGGGGDIQMTQSPSSLSASVGDRVTITCRTSRSISQYLAWYQQKPGKVPKLLIYSGSTLQSGVPSRFSGSGSGTDFTLTISSLQPEDVATYYCQQHNENPLTFGGGTKVEIKGGC

SEQ ID NO: 16 - protein, 394 aa, Artificial Sequence
  Antigen binding construct or fragment thereof
METDTLLLWVLLLWVPGSTGDVQINQSPSFLAASPGETITINCRTSRSISQYLAWYQEKPGKTNKLLIYSGSTLQSGIPSRFSGSGSGTDFTLTISGLEPEDFAMYYCQQHNENPLTFGAGTKLELKGSTSGGGSGGGSGGGGSSEVQLQQSGAELVKPGASVKLSCTASGFNIKDTYIHFVRQRPEQGLEWIGRIDPANDNTLYASKFQGKATITADTSSNTAYMHLSSLTSGDTAVYYCGRGYGYYVFDHWGQGTTLTVSSEPKSCDKTHTCPPCGGGSSGGGSGGQPREPQVYTLPPSRDELTKNQVSLTCLVKGFYPSDIAVEWESNGQPENNYKTTPPVLDSDGSFFLYSKLTVDKSRWQQGNVFSCSVMHEALHNHYTQKSLSLSPGK

SEQ ID NO: 17 - DNA, 1185 bp, Artificial Sequence
  Antigen binding construct or fragment thereof
atggagacagacaccctgctcctgtgggtgctgctcctctgggtccctggatccaccggcgatgtccagatcaaccaaagccccagctttctggctgcctcccctggagagacaatcaccatcaattgccggaccagccggagcatttcccagtacctcgcctggtaccaggaaaagcctggcaagaccaacaagctgctgatctactccggctccacactccagagcggcattccctccaggtttagcggatccggatccggaaccgacttcacactcaccatctccggcctggagcccgaggacttcgccatgtattattgccagcagcacaatgagaaccccctgaccttcggcgctggcaccaagctggagctgaaaggctccaccagcggaggcggatccggaggaggaagcggcggcggaggctcctccgaagtgcagctgcaacagagcggcgccgaactggtgaagcctggagcttccgtgaaactcagctgtaccgccagcggcttcaacatcaaggatacctacatccacttcgtgcggcaaaggcctgagcagggcctggaatggatcggcaggatcgaccccgccaacgacaacaccctctacgcctccaagttccaaggcaaggccacaatcaccgctgatacaagctccaacaccgcctacatgcacctcagctccctgaccagcggagacaccgccgtgtactactgcggacggggatacggctactatgtgttcgaccactggggccaaggcaccacactcaccgtgtcctccgagcccaagtcctgcgacaagacacacacctgtcccccttgtggaggaggatcctccggaggcggctccggcggacagcctagggagccccaggtgtacacactgcccccttccagggacgaactcaccaagaaccaggtgtccctgacctgcctggtgaagggattctaccccagcgacatcgccgtggagtgggagtccaacggccaacccgagaacaattacaagaccaccccccctgtgctcgattccgacggctccttcttcctgtactccaagctcaccgtggacaagtcccggtggcaacagggcaatgtgttctcctgcagcgtcatgcacgaggccctgcataaccactacacccagaaatccctcagcctctcccctggaaaatga

SEQ ID NO: 18 - protein, 394 aa, Artificial Sequence
  Antigen binding construct or fragment thereof
METDTLLLWVLLLWVPGSTGEVQLQQSGAELVKPGASVKLSCTASGFNIKDTYIHFVRQRPEQGLEWIGRIDPANDNTLYASKFQGKATITADTSSNTAYMHLSSLTSGDTAVYYCGRGYGYYVFDHWGQGTTLTVSSGSTSGGGSGGGSGGGGSSDVQINQSPSFLAASPGETITINCRTSRSISQYLAWYQEKPGKTNKLLIYSGSTLQSGIPSRFSGSGSGTDFTLTISGLEPEDFAMYYCQQHNENPLTFGAGTKLELKEPKSCDKTHTCPPCGGGSSGGGSGGQPREPQVYTLPPSRDELTKNQVSLTCLVKGFYPSDIAVEWESNGQPENNYKTTPPVLDSDGSFFLYSKLTVDKSRWQQGNVFSCSVMHEALHNHYTQKSLSLSPGK

SEQ ID NO: 19 - DNA, 1185 bp, Artificial Sequence
  Antigen binding construct or fragment thereof
atggagaccgacacactcctgctctgggtgctcctgctgtgggtgcctggcagcacaggagaagtgcagctgcagcagtccggcgccgaactcgtcaaacccggagcctccgtcaaactgtcctgcacagccagcggcttcaacatcaaggacacctacatccatttcgtgcggcaaaggcctgaacagggactcgagtggatcggcaggatcgaccccgccaacgacaataccctctacgcctccaagttccagggaaaggccaccattaccgccgacacatccagcaacaccgcctacatgcacctcagctccctgacatccggcgacaccgccgtgtactactgcggcaggggctacggctactacgtgtttgaccactggggccagggaacaaccctgaccgtgtccagcggctccacctccggaggcggaagcggcggaggatccggaggaggaggctcctccgacgtgcaaatcaaccagtcccctagcttcctggccgctagccctggcgagacaatcacaatcaattgtcggaccagccggtccatctcccagtatctggcctggtaccaggagaagcccggcaagacaaacaagctgctcatctacagcggcagcaccctccaatccggcatcccttcccggtttagcggctccggatccggaaccgactttaccctgaccatcagcggcctggaacccgaggatttcgccatgtactactgccagcagcacaacgagaatcccctgacctttggagccggcacaaagctcgagctgaaggagcccaagagctgcgacaaaacccacacctgtcccccttgcggaggaggatcctccggcggcggaagcggaggacaacccagggagccccaggtctacaccctgcctcctagccgggacgaactgacaaagaaccaggtgtccctgacctgtctcgtcaagggcttctacccttccgacatcgccgtcgagtgggaaagcaacggccagcccgagaacaattacaagaccacaccccccgtcctggacagcgatggcagcttcttcctctactccaagctgaccgtggacaagagccggtggcaacaaggcaacgtgttctcctgcagcgtcatgcatgaggccctgcacaatcactacacccagaagagcctgagcctctcccccggcaagtga

SEQ ID NO: 20 - protein, 394 aa, Artificial Sequence
  Antigen binding construct or fragment thereof
METDTLLLWVLLLWVPGSTGDIQMTQSPSSLSASVGDRVTITCRTSRSISQYLAWYQQKPGKVPKLLIYSGSTLQSGVPSRFSGSGSGTDFTLTISSLQPEDVATYYCQQHNENPLTFGGGTKVEIKGSTSGGGSGGGSGGGGSSQVQLVQSGAEVKKPGATVKISCKVSGFNIKDTYIHWVQQAPGKGLEWMGRIDPANDNTLYASKFQGRVTITADTSTDTAYMELSSLRSEDTAVYYCARGYGYYVFDHWGQGTLVTVSSEPKSCDKTHTCPPCGGGSSGGGSGGQPREPQVYTLPPSRDELTKNQVSLTCLVKGFYPSDIAVEWESNGQPENNYKTTPPVLDSDGSFFLYSKLTVDKSRWQQGNVFSCSVMHEALHNHYTQKSLSLSPGK

SEQ ID NO: 21 - DNA, 1185 bp, Artificial Sequence
  Antigen binding construct or fragment thereof
atggagacagacaccctcctgctgtgggtcctgctgctgtgggtgcctggcagcacaggagacatccaaatgacccagtcccctagcagcctcagcgcttccgtcggagacagggtcaccatcacatgcaggacctccaggtccatcagccagtatctggcctggtatcagcagaaacccggcaaggtgcctaagctgctgatctacagcggcagcacactccagagcggagtgcccagccggttttccggaagcggatccggaaccgacttcaccctgaccatttccagcctgcaacctgaagacgtggccacctactactgtcagcagcacaacgagaaccccctcaccttcggcggaggcaccaaagtcgagatcaagggcagcaccagcggaggaggaagcggcggaggctccggaggaggaggctcctcccaagtgcagctcgtccaaagcggcgctgaggtgaaaaagcccggcgccacagtcaaaatctcctgcaaggtcagcggcttcaacatcaaggatacctacatccactgggtgcaacaggcccccggcaaaggactcgaatggatgggccggatcgaccctgctaacgacaacacactctacgcctccaagttccagggcagggtgaccatcaccgccgatacctccaccgacacagcctacatggagctgagcagcctgaggtccgaggacaccgccgtctattactgcgcccggggatacggctactacgtgtttgaccattggggacagggaacactcgtgaccgtgagctccgagcccaagagctgcgacaagacccacacatgtcctccttgcggaggaggcagctccggaggcggatccggcggacaacctagggagccccaggtctataccctgccccccagcagggacgagctgacaaagaaccaggtctccctgacctgcctggtgaaaggattctaccccagcgacatcgctgtcgaatgggagtccaacggccagcccgagaacaactacaagacaaccccccccgtgctggattccgacggcagcttcttcctctactccaagctgaccgtcgacaagtccaggtggcagcagggcaacgtgttttcctgctccgtgatgcatgaggccctgcacaaccactacacccagaagtccctgagcctcagccctggcaagtga

SEQ ID NO: 22 - protein, 394 aa, Artificial Sequence
  Antigen binding construct or fragment thereof
METDTLLLWVLLLWVPGSTGQVQLVQSGAEVKKPGATVKISCKVSGFNIKDTYIHWVQQAPGKGLEWMGRIDPANDNTLYASKFQGRVTITADTSTDTAYMELSSLRSEDTAVYYCARGYGYYVFDHWGQGTLVTVSSGSTSGGGSGGGSGGGGSSDIQMTQSPSSLSASVGDRVTITCRTSRSISQYLAWYQQKPGKVPKLLIYSGSTLQSGVPSRFSGSGSGTDFTLTISSLQPEDVATYYCQQHNENPLTFGGGTKVEIKEPKSCDKTHTCPPCGGGSSGGGSGGQPREPQVYTLPPSRDELTKNQVSLTCLVKGFYPSDIAVEWESNGQPENNYKTTPPVLDSDGSFFLYSKLTVDKSRWQQGNVFSCSVMHEALHNHYTQKSLSLSPGK

SEQ ID NO: 23 - DNA, 1185 bp, Artificial Sequence
  Antigen binding construct or fragment thereof
atggagaccgatacactgctgctctgggtgctgctgctgtgggtgcctggaagcaccggacaggtgcaactggtccagtccggcgccgaggtgaaaaagcctggcgccaccgtcaagatctcctgtaaggtgagcggcttcaacatcaaggacacctacatccactgggtgcagcaggctcccggaaagggactggagtggatgggcaggatcgaccctgccaatgacaacaccctctacgccagcaagttccaaggacgggtgaccatcacagccgacacatccaccgacacagcctatatggagctctccagcctgaggtccgaggacaccgccgtgtactactgtgccaggggatacggctattacgtgttcgaccactggggacagggcaccctggtgaccgtgagcagcggaagcaccagcggcggaggcagcggaggcggaagcggcggcggcggatcctccgacattcagatgacccaatccccctccagcctgtccgctagcgtgggagacagggtgacaatcacatgtcggacctccaggtccatcagccaatatctcgcctggtatcagcagaagcccggcaaggtgcccaagctcctgatctacagcggctccaccctccaaagcggagtgccttcccggtttagcggaagcggcagcggcacagactttaccctgacaatcagctccctgcaacctgaggacgtcgccacatactactgccagcagcacaacgagaaccctctcacctttggcggcggcaccaaagtggagatcaaggagcccaaatcctgcgacaagacacacacctgccccccttgtggaggaggcagctccggcggcggcagcggcggacaaccccgggaacctcaggtgtatacactccccccttccagggatgagctgaccaagaaccaagtctccctgacctgtctggtgaaaggcttctacccctccgacatcgctgtcgagtgggagagcaacggccagcccgaaaacaactataagaccaccccccccgtgctcgattccgatggcagcttcttcctgtactccaagctcacagtcgacaagagccggtggcaacagggcaacgtcttctcctgtagcgtcatgcacgaggccctccacaaccactacacccagaagtccctctccctgagccccggaaaatga

SEQ ID NO: 24 - protein, 235 aa, Homo sapiens
MALPVTALLLPLALLLHAARPSQFRVSPLDRTWNLGETVELKCQVLLSNPTSGCSWLFQPRGAAASPTFLLYLSQNKPKAAEGLDTQRFSGKRLGDTFVLTLSDFRRENEGYYFCSALSNSIMYFSHFVPVFLPAKPTTTPAPRPPTPAPTIASQPLSLRPEACRPAAGGAVHTRGLDFACDIYIWAPLAGTCGVLLLSLVITLYCNHRNRRRVCKCPRPVVKSGDKPSLSARYV

SEQ ID NO: 25 - DNA, 60 bp, Artificial Sequence
  Antigen binding construct or fragment thereof
atggaaaccgacaccctgctgctgtgggtgctgctgctctgggtcccaggctccaccggt

SEQ ID NO: 26 - protein, 20 aa, Artificial Sequence
  Antigen binding construct or fragment thereof
METDTLLLWVLLLWVPGSTG

SEQ ID NO: 27 - DNA, 15 bp, Artificial Sequence
  Antigen binding construct or fragment thereof
agtggtggaggaggc

SEQ ID NO: 28 - protein, 5 aa, Artificial Sequence
  Antigen binding construct or fragment thereof
SGGGG

SEQ ID NO: 29 - DNA, 24 bp, Artificial Sequence
  Antigen binding construct or fragment thereof
ggcggagggagtggcggaggcggc

SEQ ID NO: 30 - protein, 8 aa, Artificial Sequence
  Antigen binding construct or fragment thereof
GGGSGGGG

SEQ ID NO: 31 - DNA, 9 bp, Artificial Sequence
  Antigen binding construct or fragment thereof
ggcggctgc

SEQ ID NO: 32 - protein, 3 aa, Artificial Sequence
  Antigen binding construct or fragment thereof
GGC

SEQ ID NO: 33 - DNA, 60 bp, Artificial Sequence; identical to SEQ ID NO: 25
  Antigen binding construct or fragment thereof

SEQ ID NO: 34 - protein, 20 aa, Artificial Sequence
  Antigen binding construct or fragment thereof
METDTLLLWVLLLWVPGSTG

SEQ ID NO: 35 - DNA, 54 bp, Artificial Sequence
  Antigen binding construct or fragment thereof
ggctccacatccggcggaggctctggcggtggatctggcggaggcggctcatcc

SEQ ID NO: 36 - protein, 18 aa, Artificial Sequence
  Antigen binding construct or fragment thereof
GSTSGGGSGGGSGGGGSS

SEQ ID NO: 37 - DNA, 393 bp, Artificial Sequence
  Antigen binding construct or fragment thereof
gagcctaagtcctgcgacaagacccacacctgtcccccttgcggcggaggaagcagcggaggcggatccggtggccagcctcgggagcctcaggtgtacaccctgcctccctcccgggacgagctgaccaagaaccaggtgtccctgacctgtctggtcaagggcttctacccttccgatatcgccgtggagtgggagtccaacggccagcctgagaacaactacaagaccacccctcctgtgctggactccgacggctccttcttcctgtactccaagctcacagtggataagtcccggtggcagcagggcaacgtgttctcctgctccgtgatgcacgaggccctgcacaaccactatacccagaagtccctgtccctgtctcctggcaag

SEQ ID NO: 38 - protein, 131 aa, Artificial Sequence
  Antigen binding construct or fragment thereof
EPKSCDKTHTCPPCGGGSSGGGSGGQPREPQVYTLPPSRDELTKNQVSLTCLVKGFYPSDIAVEWESNGQPENNYKTTPPVLDSDGSFFLYSKLTVDKSRWQQGNVFSCSVMHEALHNHYTQKSLSLSPGK

SEQ ID NO: 39 - DNA, 321 bp, Murine
gatgtccagataaaccagtctccatcttttcttgctgcgtctcctggagaaaccattactataaattgcaggacaagtaggagtattagtcaatatttagcctggtatcaagagaaacctgggaaaactaataagcttcttatctactctggatccactctgcaatctggaattccatcaaggttcagtggcagtggatctggtacagatttcactctcaccatcagtggcctggagcctgaagattttgcaatgtattactgtcaacagcataatgaaaacccgctcacgttcggtgctgggaccaagctggagctgaag

SEQ ID NO: 40 - protein, 107 aa, Murine; identical to SEQ ID NO: 7

SEQ ID NO: 41 - DNA, 321 bp, Artificial Sequence
  Antigen binding construct or fragment thereof
gacgtccagataacccagtctccatcctccctgtctgcatctgtaggagacagagtcaccatcacttgcaggacaagtaggagtattagtcaatatttagcctggtatcagcagaaaccagggaaagttcctaagctcctgatctattctggatccactctgcaatctggagtcccatctcggttcagtggcagtggatctgggacagatttcactctcaccatcagcagcctgcagcctgaagatgttgcaacttattactgtcaacagcataatgaaaacccgctcacgttcggcggagggaccaaggtggagatcaaa

SEQ ID NO: 42 - protein, 107 aa, Artificial Sequence; identical to SEQ ID NO: 9
  Antigen binding construct or fragment thereof

SEQ ID NO: 43 - DNA, 354 bp, Murine
gaggtccagctgcagcagtctggggcagagcttgtgaagccaggggcctcagtcaagttgtcctgcacagcttctggcttcaacattaaagacacctatatacacttcgtgaggcagaggcctgaacagggcctggagtggattggaaggattgatcctgcgaatgataatactttatatgcctcaaagttccagggcaaggccactataacagcagacacatcatccaacacagcctacatgcacctctgcagcctgacatctggggacactgccgtctattactgtggtagaggttatggttactacgtatttgaccactggggccaaggcaccactctcacagtctcctca

SEQ ID NO: 44 - protein, 118 aa, Murine; identical to SEQ ID NO: 1

SEQ ID NO: 45 - DNA, 354 bp, Artificial Sequence
  Antigen binding construct or fragment thereof
gaagtgcagctggtggaaagcggcggcggcctggtgcagccgggcggcagcctgcgcctgagctgcgcggcgagcggctttaacattaaagatacctatattcattttgtgcgccaggcgccgggcaaaggcctggaatggattggccgcattgatccggcgaacgataacaccctgtatgcgagcaaatttcagggcaaagcgaccattagcgcggataccagcaaaaacaccgcgtatctgcagatgaacagcctgcgcgcgggagataccgcggtgtattattgcggccgcggctatggctattatgtgtttgatcattggggccagggcaccctggtgaccgtgagcagc

SEQ ID NO: 46 - protein, 118 aa, Artificial Sequence
  Antigen binding construct or fragment thereof
EVQLVESGGGLVQPGGSLRLSCAASGFNIKDTYIHFVRQAPGKGLEWIGRIDPANDNTLYASKFQGKATISADTSKNTAYLQMNSLRAGDTAVYYCGRGYGYYVFDHWGQGTLVTVSS

SEQ ID NO: 47 - DNA, 354 bp, Artificial Sequence
  Antigen binding construct or fragment thereof
gaagtgcagctggtggaaagcggcggcggcctggtgcagccgggcggcagcctgcgcctgagctgcgcggcgagcggctttaacattaaagatacctatattcattttgtgcgccaggcgccgggcaaaggcctggaatggattggccgcattgatccggcgaacgataacaccctgtatgcgagcaaatttcagggcaaagcgaccattagcgcggataccagcaaaaacaccgcgtatctgcagatgaacagcctgcgcgcggaagataccgcggtgtattattgcggccgcggctatggctattatgtgtttgatcattggggccagggcaccctggtgaccgtgagcagc

SEQ ID NO: 48 - protein, 118 aa, Artificial Sequence
  Antigen binding construct or fragment thereof
EVQLVESGGGLVQPGGSLRLSCAASGFNIKDTYIHFVRQAPGKGLEWIGRIDPANDNTLYASKFQGKATISADTSKNTAYLQMNSLRAEDTAVYYCGRGYGYYVFDHWGQGTLVTVSS

SEQ ID NO: 49 - DNA, 354 bp, Artificial Sequence
  Antigen binding construct or fragment thereof
caggtgcagctggtgcagagcggcgcggaagtgaaaaaaccgggcgcgaccgtgaaaattagctgcaaagtgagcggctttaacattaaagatacctatattcattttgtgcagcaggcgccgggcaaaggcctggaatggattggccgcattgatccggcgaacgataacaccctgtatgcgagcaaatttcagggcaaagcgaccattaccgcggataccagcaccgataccgcgtatatggaactgagcagcctgcgcagcggagataccgcggtgtattattgcggccgcggctatggctattatgtgtttgatcattggggccagggcaccctggtgaccgtgagcagc

SEQ ID NO: 50 - protein, 118 aa, Artificial Sequence
  Antigen binding construct or fragment thereof
QVQLVQSGAEVKKPGATVKISCKVSGFNIKDTYIHFVQQAPGKGLEWIGRIDPANDNTLYASKFQGKATITADTSTDTAYMELSSLRSGDTAVYYCGRGYGYYVFDHWGQGTLVTVSS

SEQ ID NO: 51 - DNA, 354 bp, Artificial Sequence
  Antigen binding construct or fragment thereof
caggtgcagctggtgcagagcggcgcggaagtgaaaaaaccgggcgcgaccgtgaaaattagctgcaaagtgagcggctttaacattaaagatacctatattcattttgtgcagcaggcgccgggcaaaggcctggaatggattggccgcattgatccggcgaacgataacaccctgtatgcgagcaaatttcagggcaaagcgaccattaccgcggataccagcaccgataccgcgtatatggaactgagcagcctgcgcagcgaagataccgcggtgtattattgcggccgcggctatggctattatgtgtttgatcattggggccagggcaccctggtgaccgtgagcagc

SEQ ID NO: 52 - protein, 117 aa, Artificial Sequence
  Antigen binding construct or fragment thereof
QVQLVQSGAEVKKPGATVKISCKVSGFNIKDTYIHFVQQAPGKGLEWIGRIDPANDNTLYASKFQGKATITADTSTDTAYMELSSLRSEDTAVYYCGRGYGYYVFDHWGQGTLVTVS

SEQ ID NO: 53 - protein, 23 aa, Artificial Sequence
  Antigen binding construct or fragment thereof
EPKSCDKTHTCPPCPAPELLGGP

SEQ ID NO: 54 - protein, 25 aa, Artificial Sequence
  Antigen binding construct or fragment thereof
EPKSCDKTHTCPPCPGGGSSGGGSG

SEQ ID NO: 55 - protein, 19 aa, Artificial Sequence
  Antigen binding construct or fragment thereof
ERKCCVECPPCPAPPVAGP

SEQ ID NO: 56 - protein, 70 aa, Artificial Sequence
  Antigen binding construct or fragment thereof
ELKTPLGDTTHTCPRCPEPKSCDTPPPCPRCPEPKSCDTPPPCPRCPEPKSCDTPPPCPRCPAPELLGGP

SEQ ID NO: 57 - protein, 25 aa, Artificial Sequence
  Antigen binding construct or fragment thereof
ELKTPLGDTTHTCPRCPAPELLGGP

SEQ ID NO: 58 - protein, 23 aa, Artificial Sequence
  Antigen binding construct or fragment thereof
EPKSCDTPPPCPRCPAPELLGGP

SEQ ID NO: 59 - protein, 20 aa, Artificial Sequence
  Antigen binding construct or fragment thereof
ESKYGPPCPSCPAPEFLGGP

SEQ ID NO: 60 - protein, 20 aa, Artificial Sequence
  Antigen binding construct or fragment thereof
ESKYGPPCPPCPAPEFLGGP

SEQ ID NO: 61 - DNA, 15 bp, Artificial Sequence
  Restriction site
tctagagccgccacc

SEQ ID NO: 62 - DNA, 15 bp, Artificial Sequence
  Restriction site
tctagagccgccacc

SEQ ID NO: 63 - DNA, 6 bp, Artificial Sequence
  Restriction site
aagctt

SEQ ID NO: 64 - DNA, 6 bp, Artificial Sequence
  Restriction site
aagctt

SEQ ID NO: 65 - DNA, 15 bp, Artificial Sequence
  Restriction site
tctagagccgccacc

SEQ ID NO: 66 - DNA, 6 bp, Artificial Sequence
  Restriction site
aagctt

SEQ ID NO: 67 - DNA, 15 bp, Artificial Sequence
  Restriction site
tctagagccgccacc

SEQ ID NO: 68 - DNA, 6 bp, Artificial Sequence
  Restriction site
aagctt

SEQ ID NO: 69 - DNA, 15 bp, Artificial Sequence
  Restriction site
tctagagccgccacc

SEQ ID NO: 70 - DNA, 6 bp, Artificial Sequence
  Restriction site
aagctt

SEQ ID NO: 71 - DNA, 15 bp, Artificial Sequence
  Restriction site
tctagagccgccacc

SEQ ID NO: 72 - DNA, 6 bp, Artificial Sequence
  Restriction site
aagctt

SEQ ID NO: 73 - DNA, 15 bp, Artificial Sequence
  Restriction site
tctagagccgccacc

SEQ ID NO: 74 - DNA, 6 bp, Artificial Sequence
  Restriction site
aagctt

SEQ ID NO: 75 - DNA, 15 bp, Artificial Sequence
  Restriction site
tctagagccgccacc

SEQ ID NO: 76 - DNA, 6 bp, Artificial Sequence
  Restriction site
aagctt

SEQ ID NO: 77 - DNA, 759 bp, Artificial Sequence
  Antigen binding construct or fragment thereof
atggagaccgatacactgctgctgtgggtgctgctgctctgggtccctggcagcacaggagacatccagatgacacagagccctagctccctgagcgcttccgtgggagatagggtgaccatcacatgccggacctccaggtccatctcccagtacctggcctggtaccagcagaagcccggcaaggtgcccaagctgctcatctatagcggcagcaccctgcagagcggagtgccttcccggttttccggatccggctccggcacagactttaccctgaccatctccagcctgcagcctgaggatgtcgccacctactactgccaacagcacaacgagaaccccctgaccttcggcggcggaaccaaggtcgagatcaagtccggaggaggaggccaagtgcagctggtccaatccggcgccgaagtgaaaaagcccggcgccaccgtgaagatcagctgcaaggtgtccggcttcaacatcaaggacacctatatccactgggtccagcaagcccccggaaaaggcctggagtggatgggacggattgaccccgccaacgacaacacactctatgcctccaagttccagggcagggtgacaatcaccgccgacaccagcaccgacacagcttatatggagctgtcctccctccggtccgaggataccgccgtctactactgcgccaggggctacggctactacgtgtttgaccactggggccagggcaccctggtgacagtgtccagcggaggctgc

SEQ ID NO: 78 - DNA, 759 bp, Artificial Sequence
  Antigen binding construct or fragment thereof
atggagaccgacaccctgctgctctgggtcctcctgctgtgggtgcctggcagcacaggacaggtgcaactggtgcagagcggcgccgaggtcaagaaacctggcgccaccgtgaagatcagctgcaaggtgtccggcttcaacatcaaggacacctacatccactgggtccaacaagcccccggaaagggcctggaatggatgggccggattgaccccgccaacgacaacaccctctatgccagcaagttccagggcagggtcaccatcaccgccgacaccagcaccgacaccgcctacatggagctgagcagcctgcggagcgaagacaccgccgtgtactactgcgccaggggctacggctactacgtcttcgaccattggggacagggcaccctcgtgacagtgtccagctccggcggaggaggagatatccagatgacccagagcccttccagcctgtccgcttccgtgggagatcgggtgaccatcacatgcaggacctccaggtccatctcccagtacctggcctggtaccaacagaagcccggcaaggtgcccaagctgctgatctacagcggcagcacactgcaatccggcgtcccttcccggttttccggatccggatccggcaccgacttcaccctgaccatcagctccctgcaacccgaggacgtggccacctactactgtcagcagcacaacgagaaccccctcacctttggcggcggaaccaaggtcgagatcaagggcggctgc

SEQ ID NO: 79 - protein, 22 aa, Artificial Sequence
  Antigen binding construct or fragment thereof
ERKCCVECPPCPGGGSSGGGSG

SEQ ID NO: 80 - protein, 107 aa, Artificial Sequence
  Antigen binding construct or fragment thereof
GQPREPQVYTLPPSREEMTKNQVSLTCLVKGFYPSDIAVEWESNGQPENNYKTTPPMLDSDGSFFLYSKLTVDKSRWQQGNVFSCSVMHEALHNHYTQKSLSLSPGK

SEQ ID NO: 81 - protein, 107 aa, Artificial Sequence
  Antigen binding construct or fragment thereof
GQPREPQVYTLPPSRDELTKNQVSLTCLVKGFYPSDIAVEWESNGQPENNYKTTPPVLDSDGSFFLYSKLTVDKSRWQQGNVFSCSVMHEALHNHYTQKSLSLSPGK

SEQ ID NO: 82 - protein, 107 aa, Artificial Sequence; identical to SEQ ID NO: 9
  IAB22M variable light sequence

SEQ ID NO: 83 - protein, 18 aa, Artificial Sequence
  Linker sequence
GSTSGGGSGGGSGGGGSS

SEQ ID NO: 84 - protein, 118 aa, Artificial Sequence; identical to SEQ ID NO: 48
  IAB22M variable heavy sequence

SEQ ID NO: 85 - protein, 22 aa, Artificial Sequence
  Human IgG2 EH1
ERKCCVECPPCPGGGSSGGGSG

SEQ ID NO: 86 - protein, 3 aa, Artificial Sequence
  Upper hinge
ERK

SEQ ID NO: 87 - protein, 9 aa, Homo sapiens
CCVECPPCP

SEQ ID NO: 88 - protein, 10 aa, Homo sapiens
GGGSSGGGSG

SEQ ID NO: 89 - protein, 107 aa, Artificial Sequence; identical to SEQ ID NO: 80
  Human IgG2 CH3

SEQ ID NO: 90 - protein, 22 aa, Artificial Sequence
  Human IgG2 EH2
ERKSCVECPPCPGGGSSGGGSG

SEQ ID NO: 91 - protein, 9 aa, Homo sapiens
SCVECPPCP

SEQ ID NO: 92 - protein, 24 aa, Artificial Sequence
  Human IgG1 EH1
EPKSCDKTHTCPPCGGGSSGGGSG

SEQ ID NO: 93 - protein, 10 aa, Artificial Sequence
  Upper hinge
EPKSCDKTHT

SEQ ID NO: 94 - protein, 4 aa, Homo sapiens
CPPC

SEQ ID NO: 95 - protein, 107 aa, Artificial Sequence; identical to SEQ ID NO: 81
  Human IgG1 CH3 (G1m1 allotype)

SEQ ID NO: 96 - protein, 107 aa, Artificial Sequence
  Human IgG1 CH3 (nG1m1 allotype)
GQPREPQVYTLPPSREEMTKNQVSLTCLVKGFYPSDIAVEWESNGQPENNYKTTPPVLDSDGSFFLYSKLTVDKSRWQQGNVFSCSVMHEALHNHYTQKSLSLSPGK

SEQ ID NO: 97 - protein, 19 aa, Artificial Sequence
  Human IgG2 NH1
ERKCCVECPPCPAPPVAGP

SEQ ID NO: 98 - protein, 7 aa, Homo sapiens
APPVAGP

SEQ ID NO: 99 - protein, 19 aa, Artificial Sequence
  Human IgG2 NH2
ERKSCVECPPCPAPPVAGP

SEQ ID NO: 100 - protein, 27 aa, Artificial Sequence
  Human IgG1 EH3
EPKSSDKTHTCPPCPPCGGGSSGGGSG

SEQ ID NO: 101 - protein, 10 aa, Artificial Sequence
  Upper hinge
EPKSSDKTHT

SEQ ID NO: 102 - protein, 7 aa, Homo sapiens
CPPCPPC

SEQ ID NO: 103 - protein, 30 aa, Artificial Sequence
  Human IgG1 EH5
EPKSSDKTHTCPPCPPCPPCGGGSSGGGSG

SEQ ID NO: 104 - protein, 10 aa, Homo sapiens
CPPCPPCPPC

SEQ ID NO: 105 - protein, 10 aa, Homo sapiens
CPPCVECPPC

SEQ ID NO: 106 - protein, 29 aa, Artificial Sequence
  IgG3/IgG1 EH6
ELKTPLGDTTHTCVECPPCGGGSSGGGSG

SEQ ID NO: 107 - protein, 12 aa, Artificial Sequence
  Upper hinge
ELKTPLGDTTHT

SEQ ID NO: 108 - protein, 7 aa, Homo sapiens
CVECPPC

SEQ ID NO: 109 - protein, 29 aa, Artificial Sequence
  IgG3/IgG1 EH7
ELKTPLGDTTHTCPPCPPCGGGSSGGGSG

SEQ ID NO: 110 - protein, 32 aa, Artificial Sequence
  IgG3/IgG1 EH8
ELKTPLGDTTHTCPPCPPCPPCGGGSSGGGSG

SEQ ID NO: 111 - protein, 24 aa, Artificial Sequence
  Human IgG1 EH2
EPKSSDKTHTCPPCGGGSSGGGSG

SEQ ID NO: 112 - protein, 12 aa, Artificial Sequence
  Linker sequence
GSTSGGGSGGGS

SEQ ID NO: 113 - protein, 15 aa, Artificial Sequence
  Linker sequence
GGGGSGGGGSGGGGS

SEQ ID NO: 114 - protein, 10 aa, Artificial Sequence
  Linker sequence
GGGGSGGGGS

SEQ ID NO: 115 - protein, 5 aa, Artificial Sequence
  Linker sequence
GGGGS

SEQ ID NO: 116 - protein, 23 aa, Artificial Sequence
  Human IgG1 NH1
EPKSCDKTHTCPPCPAPELLGGP

SEQ ID NO: 117 - protein, 23 aa, Homo sapiens
  Human IgG1 NH2
EPKSSDKTHTCPPCPAPELLGGP

SEQ ID NO: 118 - protein, 25 aa, Artificial Sequence
  Human IgG1 NH3
EPKSSDKTHTCPPCPPCAPELLGGP

SEQ ID NO: 119 - protein, 28 aa, Artificial Sequence
  Human IgG1 NH4
EPKSSDKTHTCPPCVECPPCAPELLGGP

SEQ ID NO: 120 - protein, 30 aa, Artificial Sequence
  Human IgG1 EH4
EPKSSDKTHTCPPCVECPPCGGGSSGGGSG

SEQ ID NO: 121 - protein, 28 aa, Artificial Sequence
  Human IgG1 NH5
EPKSSDKTHTCPPCPPCPPCAPELLGGP

SEQ ID NO: 122 - protein, 5 aa, Homo sapiens
CPPCP

SEQ ID NO: 123 - protein, 8 aa, Homo sapiens
APELLGGP

SEQ ID NO: 124 - protein, 20 aa, Artificial Sequence
  IgG4 NH
ESKYGPPCPPCPAPEFLGGP

SEQ ID NO: 125 - protein, 22 aa, Artificial Sequence
  IgG4 EH
ESKYGPPCPPCPGGGSSGGGSG

SEQ ID NO: 126 - protein, 7 aa, Artificial Sequence
  Upper hinge
ESKYGPP

SEQ ID NO: 127 - protein, 8 aa, Homo sapiens
APEFLGGP

SEQ ID NO: 128 - protein, 107 aa, Artificial Sequence
  Human IgG3 CH3
GQPREPQVYTLPPSREEMTKNQVSLTCLVKGFYPSDIAVEWESSGQPENNYNTTPPMLDSDGSFFLYSKLTVDKSRWQQGNIFSCSVMHEALHNRFTQKSLSLSPGK

SEQ ID NO: 129 - protein, 107 aa, Artificial Sequence
  Human IgG4 CH3
GQPREPQVYTLPPSQEEMTKNQVSLTCLVKGFYPSDIAVEWESNGQPENNYKTTPPVLDSDGSFFLYSRLTVDKSRWQEGNVFSCSVMHEALHNHYTQKSLSLSLGK

SEQ ID NO: 130 - protein, 394 aa, Artificial Sequence
  IAB22M gamma 1 EH1(Minibody 1)
METDTLLLWVLLLWVPGSTGDVQITQSPSSLSASVGDRVTITCRTSRSISQYLAWYQQKPGKVPKLLIYSGSTLQSGVPSRFSGSGSGTDFTLTISSLQPEDVATYYCQQHNENPLTFGGGTKVEIKGSTSGGGSGGGSGGGGSSEVQLVESGGGLVQPGGSLRLSCAASGFNIKDTYIHFVRQAPGKGLEWIGRIDPANDNTLYASKFQGKATISADTSKNTAYLQMNSLRAEDTAVYYCGRGYGYYVFDHWGQGTLVTVSSEPKSCDKTHTCPPCGGGSSGGGSGGQPREPQVYTLPPSRDELTKNQVSLTCLVKGFYPSDIAVEWESNGQPENNYKTTPPVLDSDGSFFLYSKLTVDKSRWQQGNVFSCSVMHEALHNHYTQKSLSLSPGK

SEQ ID NO: 131 - protein, 396 aa, Artificial Sequence
  IAB22M gamma 1 EH3(Minibody 1)
METDTLLLWVLLLWVPGSTGDVQITQSPSSLSASVGDRVTITCRTSRSISQYLAWYQQKPGKVPKLLIYSGSTLQSGVPSRFSGSGSGTDFTLTISSLQPEDVATYYCQQHNENPLTFGGGTKVEIKGSTSGGGSGGGSGGGGSSEVQLVESGGGLVQPGGSLRLSCAASGFNIKDTYIHFVRQAPGKGLEWIGRIDPANDNTLYASKFQGKATISADTSKNTAYLQMNSLRAEDTAVYYCGRGYGYYVFDHWGQGTLVTVSSEPKSSDKTHTCPPCPPCGGGSSGGGSGGQPREPQVYTLPPSREEMTKNQVSLTCLVKGFYPSDIAVEWESNGQPENNYKTTPPVLDSDGSFFLYSKLTVDKSRWQQGNVFSCSVMHEALHNHYTQKSLSLSPG

SEQ ID NO: 132 - DNA, 1191 bp, Artificial Sequence
  IAB22M gamma 1 EH3(M1)
atggagaccgataccctgctgctgtgggtgctgctgctgtgggtgcccggctccacaggcgatgtgcagatcacacagagccctagcagcctgagcgccagcgtgggagatagagtcaccatcacatgcaggaccagcagaagcattagccagtacctggcctggtaccagcaaaagcccggcaaggtgcccaagctgctgatctacagcggctccaccctgcagagcggcgtgcccagcagattctccggctccggaagcggcacagactttaccctgaccatctcctccctgcagcccgaggatgtcgccacctactactgccagcagcacaacgaaaaccccctgacatttggcggcggcaccaaggtggagatcaagggcagcaccagcggtggaggaagtggaggtggaagtggaggaggcggaagcagcgaggtgcagctggtggagagtggtggaggactggtgcagcccggaggcagcctgagactgagctgtgctgcctccggattcaatatcaaggacacctacatccacttcgtgagacaggcccccggcaagggactggagtggattggaaggatcgaccccgccaacgacaacaccctgtacgccagcaaattccagggcaaggccacaatcagcgccgacaccagcaagaacaccgcctatctgcagatgaactccctgagagccgaggacacagccgtgtactactgcggcaggggctacggctattacgtgttcgaccactggggccagggcaccctggtgacagtgagcagcgaacccaagagctccgacaagacccacacctgtcccccttgccctccttgtggcggaggaagctccggaggcggaagcggaggacagcctagggagccccaggtgtataccctccccccctccagggaagagatgaccaagaaccaggtgagcctgacctgcctcgtgaagggcttttatccctccgatatcgccgtggagtgggagagcaacggccagcctgagaacaattacaagaccaccccccctgtgctggactccgatggcagcttcttcctgtattccaagctgaccgtcgacaagtccaggtggcaacagggcaacgtcttcagctgcagcgtgatgcacgaggccctgcacaatcactacacccagaagtccctctccctgagccccggctga

SEQ ID NO: 133 - protein, 399 aa, Artificial Sequence
  IAB22M gamma 1 EH5(M1)
METDTLLLWVLLLWVPGSTGDVQITQSPSSLSASVGDRVTITCRTSRSISQYLAWYQQKPGKVPKLLIYSGSTLQSGVPSRFSGSGSGTDFTLTISSLQPEDVATYYCQQHNENPLTFGGGTKVEIKGSTSGGGSGGGSGGGGSSEVQLVESGGGLVQPGGSLRLSCAASGFNIKDTYIHFVRQAPGKGLEWIGRIDPANDNTLYASKFQGKATISADTSKNTAYLQMNSLRAEDTAVYYCGRGYGYYVFDHWGQGTLVTVSSEPKSSDKTHTCPPCPPCPPCGGGSSGGGSGGQPREPQVYTLPPSREEMTKNQVSLTCLVKGFYPSDIAVEWESNGQPENNYKTTPPVLDSDGSFFLYSKLTVDKSRWQQGNVFSCSVMHEALHNHYTQKSLSLSPG

SEQ ID NO: 134 - protein, 235 aa, Homo sapiens; identical to SEQ ID NO: 24

SEQ ID NO: 135 - protein, 210 aa, Homo sapiens
MRPRLWLLLAAQLTVLHGNSVLQQTPAYIKVQTNKMVMLSCEAKISLSNMRIYWLRQRQAPSSDSHHEFLALWDSAKGTIHGEEVEQEKIAVFRDASRFILNLTSVKPEDSGIYFCMIVGSPELTFGKGTQLSVVDFLPTTAQPTKKSTLKKRVCRLPRPETQKGPLCSPVTLGLLVAGVLVLLVSLGVAMHLCCRRRRARLRFMKQFYK

SEQ ID NO: 136 - DNA, 1200 bp, Artificial Sequence
  IAB22M gamma 1 EH5(M1)
atggagacagacaccctcctcctgtgggtgctgctgctgtgggtgcccggatccaccggagacgtgcagatcacacagagccccagctccctgtccgctagcgtgggcgacagagtgaccatcacctgcaggaccagcaggagcatctcccagtacctcgcttggtaccagcagaagcctggcaaggtgcccaagctgctgatttacagcggatccaccctgcagagcggcgtgcctagcaggtttagcggcagcggatccggaacagacttcaccctgaccatcagcagcctgcagcctgaagatgtggccacctactactgtcagcagcacaacgaaaaccccctcaccttcggcggcggcacaaaggtggaaatcaagggcagcacctccggaggaggcagcggcggaggcagcggaggcggcggctccagcgaagtgcagctggtcgagagcggaggcggactggtgcaacccggaggaagcctgaggctgagctgtgccgccagcggcttcaacatcaaggacacatacattcactttgtgaggcaggctcctggaaagggcctggagtggatcggcagaatcgaccccgctaacgacaacaccctgtacgccagcaagttccagggcaaggccaccatctccgccgacacaagcaagaataccgcctacctgcagatgaactccctgagggccgaggataccgccgtgtactactgcggcaggggctatggctactacgtgtttgaccactggggccagggcacactggtgacagtgagctccgagcccaagagctccgacaagacacacacctgccctccttgccccccttgtcctccctgtggaggaggaagcagcggaggaggaagcggcggacagcccagagagcctcaagtgtataccctgcccccctccagggaagagatgaccaagaaccaggtgagcctgacatgcctggtcaaaggcttctaccccagcgatattgctgtggagtgggagagcaacggccagcccgagaacaactacaagaccacaccccccgtcctggatagcgatggcagcttcttcctgtacagcaagctgaccgtggacaagtccaggtggcagcagggcaacgtcttctcctgcagcgtgatgcacgaggctctgcataaccactacacacagaagtccctcagcctgagccctggatga

SEQ ID NO: 137 - protein, 398 aa, Artificial Sequence
  IAB22M gamma 1 EH7(Minibody 1)
METDTLLLWVLLLWVPGSTGDVQITQSPSSLSASVGDRVTITCRTSRSISQYLAWYQQKPGKVPKLLIYSGSTLQSGVPSRFSGSGSGTDFTLTISSLQPEDVATYYCQQHNENPLTFGGGTKVEIKGSTSGGGSGGGSGGGGSSEVQLVESGGGLVQPGGSLRLSCAASGFNIKDTYIHFVRQAPGKGLEWIGRIDPANDNTLYASKFQGKATISADTSKNTAYLQMNSLRAEDTAVYYCGRGYGYYVFDHWGQGTLVTVSSELKTPLGDTTHTCPPCPPCGGGSSGGGSGGQPREPQVYTLPPSREEMTKNQVSLTCLVKGFYPSDIAVEWESNGQPENNYKTTPPVLDSDGSFFLYSKLTVDKSRWQQGNVFSCSVMHEALHNHYTQKSLSLSPG

SEQ ID NO: 138 - DNA, 1197 bp, Artificial Sequence
  IAB22M gamma 1 EH7(Minibody 1)
atggagacagacaccctcctcctgtgggtgctgctgctgtgggtgcccggatccaccggagacgtgcagatcacacagagccccagctccctgtccgctagcgtgggcgacagagtgaccatcacctgcaggaccagcaggagcatctcccagtacctcgcttggtaccagcagaagcctggcaaggtgcccaagctgctgatttacagcggatccaccctgcagagcggcgtgcctagcaggtttagcggcagcggatccggaacagacttcaccctgaccatcagcagcctgcagcctgaagatgtggccacctactactgtcagcagcacaacgaaaaccccctcaccttcggcggcggcacaaaggtggaaatcaagggcagcacctccggaggaggcagcggcggaggcagcggaggcggcggctccagcgaagtgcagctggtcgagagcggaggcggactggtgcaacccggaggaagcctgaggctgagctgtgccgccagcggcttcaacatcaaggacacatacattcactttgtgaggcaggctcctggaaagggcctggagtggatcggcagaatcgaccccgctaacgacaacaccctgtacgccagcaagttccagggcaaggccaccatctccgccgacacaagcaagaataccgcctacctgcagatgaactccctgagggccgaggataccgccgtgtactactgcggcaggggctatggctactacgtgtttgaccactggggccagggcacactggtgacagtgagctccgagctgaagacacctctgggcgacacaacacacacctgccccccttgtcctccctgtggaggaggaagcagcggaggaggaagcggcggacagcccagagagcctcaagtgtataccctgcccccctccagggaagagatgaccaagaaccaggtgagcctgacatgcctggtcaaaggcttctaccccagcgatattgctgtggagtgggagagcaacggccagcccgagaacaactacaagaccacaccccccgtcctggatagcgatggcagcttcttcctgtacagcaagctgaccgtggacaagtccaggtggcagcagggcaacgtcttctcctgcagcgtgatgcacgaggctctgcataaccactacacacagaagtccctcagcctgagccctggatga

SEQ ID NO: 139 - protein, 401 aa, Artificial Sequence
  IAB22M gamma 1 EH8(Minibody 1)
METDTLLLWVLLLWVPGSTGDVQITQSPSSLSASVGDRVTITCRTSRSISQYLAWYQQKPGKVPKLLIYSGSTLQSGVPSRFSGSGSGTDFTLTISSLQPEDVATYYCQQHNENPLTFGGGTKVEIKGSTSGGGSGGGSGGGGSSEVQLVESGGGLVQPGGSLRLSCAASGFNIKDTYIHFVRQAPGKGLEWIGRIDPANDNTLYASKFQGKATISADTSKNTAYLQMNSLRAEDTAVYYCGRGYGYYVFDHWGQGTLVTVSSELKTPLGDTTHTCPPCPPCPPCGGGSSGGGSGGQPREPQVYTLPPSREEMTKNQVSLTCLVKGFYPSDIAVEWESNGQPENNYKTTPPVLDSDGSFFLYSKLTVDKSRWQQGNVFSCSVMHEALHNHYTQKSLSLSPG

SEQ ID NO: 140 - DNA, 1206 bp, Artificial Sequence
  IAB22M gamma 1 EH8(Minibody 1)
atggagacagacaccctcctcctgtgggtgctgctgctgtgggtgcccggatccaccggagacgtgcagatcacacagagccccagctccctgtccgctagcgtgggcgacagagtgaccatcacctgcaggaccagcaggagcatctcccagtacctcgcttggtaccagcagaagcctggcaaggtgcccaagctgctgatttacagcggatccaccctgcagagcggcgtgcctagcaggtttagcggcagcggatccggaacagacttcaccctgaccatcagcagcctgcagcctgaagatgtggccacctactactgtcagcagcacaacgaaaaccccctcaccttcggcggcggcacaaaggtggaaatcaagggcagcacctccggaggaggcagcggcggaggcagcggaggcggcggctccagcgaagtgcagctggtcgagagcggaggcggactggtgcaacccggaggaagcctgaggctgagctgtgccgccagcggcttcaacatcaaggacacatacattcactttgtgaggcaggctcctggaaagggcctggagtggatcggcagaatcgaccccgctaacgacaacaccctgtacgccagcaagttccagggcaaggccaccatctccgccgacacaagcaagaataccgcctacctgcagatgaactccctgagggccgaggataccgccgtgtactactgcggcaggggctatggctactacgtgtttgaccactggggccagggcacactggtgacagtgagctccgagctgaagacacctctgggcgacacaacacacacctgccctccttgccccccttgtcctccctgtggaggaggaagcagcggaggaggaagcggcggacagcccagagagcctcaagtgtataccctgcccccctccagggaagagatgaccaagaaccaggtgagcctgacatgcctggtcaaaggcttctaccccagcgatattgctgtggagtgggagagcaacggccagcccgagaacaactacaagaccacaccccccgtcctggatagcgatggcagcttcttcctgtacagcaagctgaccgtggacaagtccaggtggcagcagggcaacgtcttctcctgcagcgtgatgcacgaggctctgcataaccactacacacagaagtccctcagcctgagccctggatga

SEQ ID NO: 141 - protein, 391 aa, Artificial Sequence
  IAB22M gamma 2 EH2(Minibody 1)
METDTLLLWVLLLWVPGSTGDVQITQSPSSLSASVGDRVTITCRTSRSISQYLAWYQQKPGKVPKLLIYSGSTLQSGVPSRFSGSGSGTDFTLTISSLQPEDVATYYCQQHNENPLTFGGGTKVEIKGSTSGGGSGGGSGGGGSSEVQLVESGGGLVQPGGSLRLSCAASGFNIKDTYIHFVRQAPGKGLEWIGRIDPANDNTLYASKFQGKATISADTSKNTAYLQMNSLRAEDTAVYYCGRGYGYYVFDHWGQGTLVTVSSERKSCVECPPCPGGGSSGGGSGGQPREPQVYTLPPSREEMTKNQVSLTCLVKGFYPSDIAVEWESNGQPENNYKTTPPMLDSDGSFFLYSKLTVDKSRWQQGNVFSCSVMHEALHNHYTQKSLSLSPG

SEQ ID NO: 142 - DNA, 1236 bp, Artificial Sequence
  IAB22M gamma 2 EH2(Minibody 1)
atggaaaccgacacactgctgctgtgggtgctgctgctgtgggtccctggctccaccggagacgtccagatcacacagagccccagcagcctgtccgccagcgtgggagacagggtgaccgacgtccagatcacacagagccccagcagcctgtccgccagcgtgggagacagggtgaccgacgtccagatcacacagagccccagcagcctgtccgccagcgtgggagacagggtgaccggcaaggtccccaaactgctgatctacagcggctccaccctgcagtccggcgtgcctagcaggttctccggcagcggatccggcaccgacttcaccctgaccatcagctccctgcagcctgaggacgtggctacctactactgccaacagcacaacgagaaccccctgacctttggaggcggcaccaaggtggaaatcaagggcagcaccagcggcggaggaagcggaggaggatccggaggaggcggaagctccgaggtgcagctggtggaaagcggcggcggactggtgcagcctggaggaagcctcagactgagctgtgccgccagcggattcaacatcaaagacacctacattcatttcgtgagacaggcccccggcaagggcctcgaatggatcggaaggatcgaccccgctaacgacaataccctgtacgcctccaagttccagggaaaggccaccatctccgccgatacctccaagaacaccgcctacctccagatgaactccctgagggccgaagataccgccgtctactactgtggcaggggctacggctactatgtgttcgatcactggggccaaggaaccctggtgaccgtgagcagcgaaaggaagagctgcgtggagtgtcctccttgtcccggcggcggctccagcggcggaggctccggcggccagcctagagaacctcaggtgtacaccctccccccctccagagaggagatgaccaagaaccaggtgtccctgacctgcctggtgaaaggcttctatcccagcgacatcgccgtggaatgggagtccaacggccagcccgagaacaactacaagaccacccctcccatgctggattccgacggcagctttttcctgtacagcaagctcaccgtggacaagagcagatggcagcagggcaacgtgttcagctgcagcgtgatgcacgaggctctgcataaccactacacccagaagagcctgtccctgtcccccggatga

SEQ ID NO: 143 - protein, 391 aa, Artificial Sequence
  IAB22M gamma 2 EH2(Minibody 1)(VH-K67R)
METDTLLLWVLLLWVPGSTGDVQITQSPSSLSASVGDRVTITCRTSRSISQYLAWYQQKPGKVPKLLIYSGSTLQSGVPSRFSGSGSGTDFTLTISSLQPEDVATYYCQQHNENPLTFGGGTKVEIKGSTSGGGSGGGSGGGGSSEVQLVESGGGLVQPGGSLRLSCAASGFNIKDTYIHFVRQAPGKGLEWIGRIDPANDNTLYASKFQGRATISADTSKNTAYLQMNSLRAEDTAVYYCGRGYGYYVFDHWGQGTLVTVSSERKSCVECPPCPGGGSSGGGSGGQPREPQVYTLPPSREEMTKNQVSLTCLVKGFYPSDIAVEWESNGQPENNYKTTPPMLDSDGSFFLYSKLTVDKSRWQQGNVFSCSVMHEALHNHYTQKSLSLSPG

SEQ ID NO: 144 - DNA, 1176 bp, Artificial Sequence
  IAB22M gamma 2 EH2(Minibody 1)
atggagaccgacaccctcctcctgtgggtgctgctgctgtgggtgcctggaagcaccggcgatgtgcagatcacccagagccctagcagcctgtccgcttccgtgggcgacagggtgaccatcacctgtaggacctccaggagcatctcccagtacctggcctggtaccagcagaagcccggcaaggtgcccaaactgctcatctactccggcagcacactccagagcggcgtccctagcagattcagcggaagcggcagcggcaccgacttcaccctgaccatcagctccctgcagcccgaggacgtggccacctattactgtcagcagcacaacgaaaaccccctgaccttcggcggcggcacaaaagtggagatcaagggcagcaccagcggaggcggatccggcggcggcagcggcggcggaggatccagcgaagtgcagctggtcgaaagcggaggcggactggtgcagcctggaggaagcctgagactcagctgcgccgcctccggattcaacatcaaggacacctacatccacttcgtgaggcaggctcccggcaaaggcctcgagtggattggaaggattgaccccgccaacgacaacaccctgtacgccagcaagttccaaggaagggccaccatctccgccgacaccagcaagaataccgcctacctgcagatgaactccctgagggctgaggacaccgccgtgtactactgcggcagaggctacggctactacgtgttcgaccactggggacagggcacactggtgacagtgagcagcgagaggaaaagctgcgtggagtgccccccctgccctggcggcggcagctccggcggaggaagcggaggacaacccagggagccccaggtgtacacactcccccctagcagggaagagatgaccaagaaccaggtgtccctgacctgcctcgtgaagggattctaccccagcgacattgccgtcgagtgggagagcaacggccagcctgagaacaactacaagacaaccccccctatgctcgatagcgatggctccttcttcctgtactccaagctcaccgtcgacaagagcaggtggcagcagggcaacgtcttctcctgtagcgtgatgcacgaggctctgcacaaccactacacccagaagagcctgagcctgagccccggctga

SEQ ID NO: 145 - protein, 118 aa, Artificial Sequence
  IAB22M variable heavy (VH-K67R) sequence
EVQLVESGGGLVQPGGSLRLSCAASGFNIKDTYIHFVRQAPGKGLEWIGRIDPANDNTLYASKFQGRATISADTSKNTAYLQMNSLRAEDTAVYYCGRGYGYYVFDHWGQGTLVTVSS

SEQ ID NO: 146 - protein, 22 aa, Artificial Sequence
  IgG4 EH
ESKYGPPCPPCPGGGSSGGGSG

SEQ ID NO: 147 - protein, 376 aa, Artificial Sequence
  IAB22 (CD8)
DVQITQSPSSLSASVGDRVTITCRTSRSISQYLAWYQQKPGKVPKLLIYSGSTLQSGVPSRFSGSGSGTDFTLTISSLQPEDVATYYCQQHNENPLTFGGGTKVEIKGSTSGGGSGGGSGGGGSSEVQLVESGGGLVQPGGSLRLSCAASGFNIKDTYIHFVRQAPGKGLEWIGRIDPANDNTLYASKFQGKATISADTSKNTAYLQMNSLRAEDTAVYYCGRGYGYYVFDHWGQGTLVTVSSEPKSSDKTHTCPPCPPCGGGSSGGGSGGQPREPQVYTLPPSREEMTKNQVSLTCLVKGFYPSDIAVEWESNGQPENNYKTTPPVLDSDGSFFLYSKLTVDKSRWQQGNVFSCSVMHEALHNHYTQKSLSLSPG